European Patent Application EP 4 647 495 A1, published November 12, 2025. Title: TRUNCATED INSULATOR AND APPLICATION THEREOF. Applicant: SHANGHAI QILU PHARMACEUTICAL RESEARCH AND DEVELOPMENT CENTRE LTD. Application US. The sequence listing filed with the application follows.

SEQUENCE LISTING (4 sequences)

SEQ ID NO: 1 - DNA, 521 bp, synthetic construct
  source 1..521: mol_type = other DNA
cggggacagcccccccccaaagcccccagggatgtaattacgtccctcccccgctagggggcagcagcgagccgcccggggctccgctccggtccggcgctccccccgcatccccgagccggcagcgtgcggggacagcccgggcacggggaaggtggcacgggatcgctttcctctgaacgcttctcgctgctctttgagcctgcagacacctggggggatacggggaaaatgtgtctgagcctgcatgtttgatggtgtctggatgcaagcagaaggggtggaagagcttgcctggagagatacagctgggtcagtaggactgggacaggcagctatccccaagaccaaccccaacccacccaccgtgcccactggccatgtccttcatcacctccagggacggtgacccccccacctccgtgggcagctgtgccactgcagcaccgctctttggagaaggtaaatcttgctaaatccagcccgaccctcccctggcacaacgtaaggccattatctct

SEQ ID NO: 2 - DNA, 490 bp, synthetic construct
  source 1..490: mol_type = other DNA
cggggacagcccccccccaaagcccccagggatgtaattacgtccctcccccgctagggggcagcagcgagccgcccggggctccgctccggtccggcgctccccccgcatccccgagccggcagcgtgcggggacagcccgggcacggggaaggtggcacgggatcgagcctgcagacacctggggggatacggggaaaatgtgtctgagcctgcatgtttgatggtgtctggatgcaagcagaaggggtggaagagcttgcctggagagatacagctgggtcagtaggactgggacaggcagctatccccaagaccaaccccaacccacccaccgtgcccactggccatgtccttcatcacctccagggacggtgacccccccacctccgtgggcagctgtgccactgcagcaccgctctttggagaaggtaaatcttgctaaatccagcccgaccctcccctggcacaacgtaaggccattatctct

SEQ ID NO: 3 - DNA, 479 bp, synthetic construct
  source 1..479: mol_type = other DNA
cggggacagcccccccccaaagcccccagggatgtaattacgtccctcccccgctagggggcagcagcgagccgcccggggctccgctccggtccggcgctccccccgcatccccgagccggcagcgtgcggggacagcccgggcacggggaaggtggcacgggatcgctttcctctgaacgcttctcgctgctctttgagcctgcagacacctggggggatgatgcaagcagaaggggtggaagagcttgcctggagagatacagctgggtcagtaggactgggacaggcagctatccccaagaccaaccccaacccacccaccgtgcccactggccatgtccttcatcacctccagggacggtgacccccccacctccgtgggcagctgtgccactgcagcaccgctctttggagaaggtaaatcttgctaaatccagcccgaccctcccctggcacaacgtaaggccattatctct

SEQ ID NO: 4 - DNA, 448 bp, synthetic construct
  source 1..448: mol_type = other DNA
cggggacagcccccccccaaagcccccagggatgtaattacgtccctcccccgctagggggcagcagcgagccgcccggggctccgctccggtccggcgctccccccgcatccccgagccggcagcgtgcggggacagcccgggcacggggaaggtggcacgggatcgagcctgcagacacctggggggatgatgcaagcagaaggggtggaagagcttgcctggagagatacagctgggtcagtaggactgggacaggcagctatccccaagaccaaccccaacccacccaccgtgcccactggccatgtccttcatcacctccagggacggtgacccccccacctccgtgggcagctgtgccactgcagcaccgctctttggagaaggtaaatcttgctaaatccagcccgaccctcccctggcacaacgtaaggccattatctct